European Patent Application EP 4 328 242 A1, published February 28, 2024. Title: Antibody specifically binding to angiopoietin-2, or its fragment. Applicant: NEORTESBIO Inc. The sequence listing filed with the application follows.

SEQUENCE LISTING (33 sequences)

SEQ ID NO: 1 - protein, 496 aa, Homo sapiens
MWQIVFFTLSCDLVLAAAYNNFRKSMDSIGKKQYQVQHGSCSYTFLLPEMDNCRSSSSPYVSNAVQRDAPLEYDDSVQRLQVLENIMENNTQWLMKLENYIQDNMKKEMVEIQQNAVQNQTAVMIEIGTNLLNQTAEQTRKLTDVEAQVLNQTTRLELQLLEHSLSTNKLEKQILDQTSEINKLQDKNSFLEKKVLAMEDKHIIQLQSIKEEKDQLQVLVSKQNSIIEELEKKIVTATVNNSVLQKQQHDLMETVNNLLTMMSTSNSAKDPTVAKEEQISFRDCAEVFKSGHTTNGIYTLTFPNSTEEIKAYCDMEAGGGGWTIIQRREDGSVDFQRTWKEYKVGFGNPSGEYWLGNEFVSQLTNQQRYVLKIHLKDWEGNEAYSLYEHFYLSSEELNYRIHLKGLTGTAGKISSISQPGNDFSTKDGDNDKCICKCSQMLTGGWWFDACGPSNLNGMYYPQRQNTNKFNGIKWYYWKGSGYSLKATTMMIRPADF

SEQ ID NO: 2 - protein, 5 aa, Artificial Sequence
  CDRH1
DYWIG

SEQ ID NO: 3 - protein, 17 aa, Artificial Sequence
  CDRH2
DIYPGGGYTNCNEKFKG

SEQ ID NO: 4 - protein, 11 aa, Artificial Sequence
  CDRH3
SDYRNDEGFAD

SEQ ID NO: 5 - protein, 12 aa, Artificial Sequence
  CDRL1
SASSSVSSSYLH

SEQ ID NO: 6 - protein, 7 aa, Artificial Sequence
  CDRL2
RTSNLAS

SEQ ID NO: 7 - protein, 9 aa, Artificial Sequence
  CDRL3
QQWSGYPYT

SEQ ID NO: 8 - protein, 122 aa, Artificial Sequence
  VH
QVQLQQSGAELVRPGTSVKMSCKAAGYTFTDYWIGWVKQRPGHGLEWIGDIYPGGGYTNCNEKFKGKATLTADTSSSTAYMQLSSLTSEDSAIYYCSRSDYRNDEGFADWGQGTLVTVSAAK

SEQ ID NO: 9 - protein, 117 aa, Artificial Sequence
  VL
ENVLTQSPAIMTASLGQKVTMTCSASSSVSSSYLHWYQQKSGASPKPLIHRTSNLASGVPARFSGSGSGTSYSLTISSVEAEDDATYYCQQWSGYPYTFGGGTKLEIKRADAAPTVS

SEQ ID NO: 10 - protein, 5 aa, Artificial Sequence
  CDRH1
NYWIG

SEQ ID NO: 11 - protein, 17 aa, Artificial Sequence
  CDRH2
DIYPGGGYTNYNEKFKG

SEQ ID NO: 12 - protein, 11 aa, Artificial Sequence
  CDRH3
SDYRDDEGFAY

SEQ ID NO: 13 - protein, 12 aa, Artificial Sequence
  CDRL1
SASSSVSSSYLH

SEQ ID NO: 14 - protein, 7 aa, Artificial Sequence
  CDRL2
RTSNLAS

SEQ ID NO: 15 - protein, 9 aa, Artificial Sequence
  CDRL3
QQWSGYPYT

SEQ ID NO: 16 - protein, 132 aa, Artificial Sequence
  VH
QVHLQQSGAELVRPGTSVKMSCKAAGYTFTNYWIGWVKQRPGHGLEWIGDIYPGGGYTNYNEKFKGKATLTADTSSSTAYMQLSSLTSEDSAIYYCSRSDYRDDEGFAYWGQGTLVTVSAAKTTPPKLYPLA

SEQ ID NO: 17 - protein, 123 aa, Artificial Sequence
  VL
ENVLTQSPAIMAASLGQKVTMTCSASSSVSSSYLHWYQQKSGASPKPLIHRTSNLASGVPARFSGSGSGTSYSLTISTVEAEDAATYYCQQWSGYPYTFGGGTKLEIKRADAAPTVSAAASLS

SEQ ID NO: 18 - protein, 6 aa, Artificial Sequence
  CDRH1
SDYGWN

SEQ ID NO: 19 - protein, 16 aa, Artificial Sequence
  CDRH2
YISYSGTTSYNPSLKS

SEQ ID NO: 20 - protein, 11 aa, Artificial Sequence
  CDRH3
SEGTGFYAMDY

SEQ ID NO: 21 - protein, 11 aa, Artificial Sequence
  CDRL1
KASQSVSNDVA

SEQ ID NO: 22 - protein, 7 aa, Artificial Sequence
  CDRL2
YASNRYT

SEQ ID NO: 23 - protein, 8 aa, Artificial Sequence
  CDRL3
QQDYSSPT

SEQ ID NO: 24 - protein, 129 aa, Artificial Sequence
  VH
DVQLQESGPGLVKPSQSLSLTCTVTGYSITSDYGWNWIRQFPGNKLEWMGYISYSGTTSYNPSLKSRISITRDTSKNQFFLQLNSVTTEDTATYYCARSEGTGFYAMDYWGQGTSVTVSSAKTTPPKLY

SEQ ID NO: 25 - protein, 108 aa, Artificial Sequence
  VL
SIVMTQTPKFLLVSAGDRVTIICKASQSVSNDVAWYQQKPGQSPKLLIYYASNRYTGVPDRFTGSGYGTDFTFTISTVQAEDLAVYFCQQDYSSPTFGGGTKLEIKRA

SEQ ID NO: 26 - protein, 5 aa, Artificial Sequence
  CDRH1
NYWIG

SEQ ID NO: 27 - protein, 15 aa, Artificial Sequence
  CDRH2
IYPGGGYTNYNEKFK

SEQ ID NO: 28 - protein, 11 aa, Artificial Sequence
  CDRH3
SDYRFDEGFAY

SEQ ID NO: 29 - protein, 12 aa, Artificial Sequence
  CDRL1
SASSSVSSSYLH

SEQ ID NO: 30 - protein, 7 aa, Artificial Sequence
  CDRL2
RTSNLAS

SEQ ID NO: 31 - protein, 9 aa, Artificial Sequence
  CDRL3
QQWSGYPYT

SEQ ID NO: 32 - protein, 119 aa, Artificial Sequence
  VH
QVQLQQSGAELVRPGTSVKMSCKATGYTFTNYWIGWVKQRPGHGLEWIGDIYPGGGYTNYNEKFKGKATLTADTSSSTACMQLSSLTSEDSAIYYCARSDYRFDEGFAYWGQGTLVTIS

SEQ ID NO: 33 - protein, 110 aa, Artificial Sequence
  VL
ENVLTQSPAIMAASLGQKVTMTCSASSSVSSSYLHWYQQKSGASPKPLIHRTSNLASGVPARFSGSGSGTSYSLTISSVEAEDDATYYCQQWSGYPYTFGGGTKLEIKRA